European Patent Application EP 4 541 820 A1, published April 23, 2025. Title: MONOCLONAL ANTIBODY AGAINST TFPI AND USE THEREOF. Applicant: AMPSOURCE BIOPHARMA SHANGHAI INC. The sequence listing filed with the application follows.

SEQUENCE LISTING (24 sequences)

SEQ ID NO: 1 - protein, 5 aa, synthetic construct
  source 1..5: note = HCDR1
SYWMH

SEQ ID NO: 2 - protein, 17 aa, synthetic construct
  source 1..17: note = HCDR2
EIKPDNGRINYNEKFKT

SEQ ID NO: 3 - protein, 10 aa, synthetic construct
  source 1..10: note = HCDR3
SSVVDVAMDY

SEQ ID NO: 4 - protein, 12 aa, synthetic construct
  source 1..12: note = LCDR1
SASSSVSSSYLY

SEQ ID NO: 5 - protein, 7 aa, synthetic construct
  source 1..7: note = LCDR2
GTSILAS

SEQ ID NO: 6 - protein, 9 aa, synthetic construct
  source 1..9: note = LCDR3
HQWSHYPFT

SEQ ID NO: 7 - protein, 8 aa, synthetic construct
  source 1..8: note = HCDR1
GYTFTSYW

SEQ ID NO: 8 - protein, 8 aa, synthetic construct
  source 1..8: note = HCDR2
IKPDNGRI

SEQ ID NO: 9 - protein, 12 aa, synthetic construct
  source 1..12: note = HCDR3
ARSSVVDVAMDY

SEQ ID NO: 10 - protein, 7 aa, synthetic construct
  source 1..7: note = LCDR1
SSVSSSY

SEQ ID NO: 11 - skipped

SEQ ID NO: 12 - protein, 17 aa, synthetic construct
  source 1..17: note = HCDR2
EIKPDQGRINYNEKFKT

SEQ ID NO: 13 - protein, 8 aa, synthetic construct
  source 1..8: note = HCDR2
IKPDQGRI

SEQ ID NO: 14 - protein, 119 aa, synthetic construct
  source 1..119: note = mAb3-71_VH
QVQLQQPEAELMKPGASVKLSCKASGYTFTSYWMHWVKQRPGQGLEWIGEIKPDNGRINYNEKFKTKATLAVDKSSSTAYMQLNSLTSGDSAVYYCARSSVVDVAMDYWGQGTSVSVSS

SEQ ID NO: 15 - protein, 108 aa, synthetic construct
  source 1..108: note = mAb3-71_VL
QIVLTQSPAIMSASPGEKVTLTCSASSSVSSSYLYWYQQKPGSSPKLWISGTSILASGVPARFSGSGSGTSYSLTISSMEAEDTASYFCHQWSHYPFTFGSGTKLEIK

SEQ ID NO: 16 - protein, 119 aa, synthetic construct
  source 1..119: note = AB8D_VH
EVQLVQSGAELKKPGASVKLSCKASGYTFTSYWMHWVRQTPGQGLEWIGEIKPDQGRINYNEKFKTRATLTADKSTSTAYMELSSLRSEDTAVYYCARSSVVDVAMDYWGQGTTVTVSS

SEQ ID NO: 17 - protein, 108 aa, synthetic construct
  source 1..108: note = AB8D_VL
EIVLTQSPATLSLSPGERATLSCSASSSVSSSYLYWYQQKPGQAPRLWISGTSILASGVPARFSGSGSGTKYTLTISSLEPEDFAVYFCHQWSHYPFTFGQGTKLEIK

SEQ ID NO: 18 - protein, 107 aa, Homo sapiens [sequence omitted]

SEQ ID NO: 19 - protein, 330 aa, Homo sapiens [sequence omitted]

SEQ ID NO: 20 - protein, 330 aa, synthetic construct
  source 1..330: note = Amino acid sequence of human IgG1 mutant
ASTKGPSVFPLAPSSKSTSGGTAALGCLVKDYFPEPVTVSWNSGALTSGVHTFPAVLQSSGLYSLSSVVTVPSSSLGTQTYICNVNHKPSNTKVDKKVEPKSCDKTHTCPPCPAPELLGGPSVFLFPPKPKDTLYITREPEVTCVVVDVSHEDPEVKFNWYVDGVEVHNAKTKPREEQYNSTYRVVSVLTVLHQDWLNGKEYKCKVSNKALPAPIEKTISKAKGQPREPQVYTLPPSRDELTKNQVSLTCLVKGFYPSDIAVEWESNGQPENNYKTTPPVLDSDGSFFLYSKLTVDKSRWQQGNVFSCSVLHEALHNHYTQKSLSLSPGK

SEQ ID NO: 21 - protein, 326 aa, Homo sapiens
ASTKGPSVFPLAPCSRSTSESTAALGCLVKDYFPEPVTVSWNSGALTSGVHTFPAVLQSSGLYSLSSVVTVPSSNFGTQTYTCNVDHKPSNTKVDKTVERKCCVECPPCPAPPVAGPSVFLFPPKPKDTLMISRTPEVTCVVVDVSHEDPEVQFNWYVDGVEVHNAKTKPREEQFNSTFRVVSVLTVVHQDWLNGKEYKCKVSNKGLPAPIEKTISKTKGQPREPQVYTLPPSREEMTKNQVSLTCLVKGFYPSDISVEWESNGQPENNYKTTPPMLDSDGSFFLYSKLTVDKSRWQQGNVFSCSVMHEALHNHYTQKSLSLSPGK

SEQ ID NO: 22 - protein, 327 aa, synthetic construct
  source 1..327: note = Amino acid sequence of human IgG4 mutant
ASTKGPSVFPLAPCSRSTSESTAALGCLVKDYFPEPVTVSWNSGALTSGVHTFPAVLQSSGLYSLSSVVTVPSSSLGTKTYTCNVDHKPSNTKVDKRVESKYGPPCPPCPAPEFLGGPSVFLFPPKPKDTLMISRTPEVTCVVVDVSQEDPEVQFNWYVDGVEVHNAKTKPREEQFNSTYRVVSVLTVLHQDWLNGKEYKCKVSNKGLPSSIEKTISKAKGQPREPQVYTLPPSQEEMTKNQVSLTCLVKGFYPSDIAVEWESNGQPENNYKTTPPVLDSDGSFFLYSRLTVDKSRWQEGNVFSCSVMHEALHNHYTQKSLSLSLGK

SEQ ID NO: 23 - protein, 446 aa, synthetic construct
  source 1..446: note = AB8D_HC
EVQLVQSGAELKKPGASVKLSCKASGYTFTSYWMHWVRQTPGQGLEWIGEIKPDQGRINYNEKFKTRATLTADKSTSTAYMELSSLRSEDTAVYYCARSSVVDVAMDYWGQGTTVTVSSASTKGPSVFPLAPCSRSTSESTAALGCLVKDYFPEPVTVSWNSGALTSGVHTFPAVLQSSGLYSLSSVVTVPSSSLGTKTYTCNVDHKPSNTKVDKRVESKYGPPCPPCPAPEFLGGPSVFLFPPKPKDTLMISRTPEVTCVVVDVSQEDPEVQFNWYVDGVEVHNAKTKPREEQFNSTYRVVSVLTVLHQDWLNGKEYKCKVSNKGLPSSIEKTISKAKGQPREPQVYTLPPSQEEMTKNQVSLTCLVKGFYPSDIAVEWESNGQPENNYKTTPPVLDSDGSFFLYSRLTVDKSRWQEGNVFSCSVMHEALHNHYTQKSLSLSLGK

SEQ ID NO: 24 - protein, 215 aa, synthetic construct
  source 1..215: note = AB8D_LC
EIVLTQSPATLSLSPGERATLSCSASSSVSSSYLYWYQQKPGQAPRLWISGTSILASGVPARFSGSGSGTKYTLTISSLEPEDFAVYFCHQWSHYPFTFGQGTKLEIKRTVAAPSVFIFPPSDEQLKSGTASVVCLLNNFYPREAKVQWKVDNALQSGNSQESVTEQDSKDSTYSLSSTLTLSKADYEKHKVYACEVTHQGLSSPVTKSFNRGEC